European Patent Application EP 4 269 576 A1, published November 1, 2023. Title: Lipase Mutant and use thereof. Applicant: ASYMECHEM LIFE SCIENCE (TIANJIN) CO., LTD. Application 21918767.1. The sequence listing filed with the application follows.

SEQUENCE LISTING (2 sequences)

SEQ ID NO: 1 - protein, 318 aa, Pseudomonas putida
MLPSGSDPAFSQPKSVLDAGLTCQGASPSSVSKPILLVPGTGTTGPQSFDSNWIPLSTQLGYTPCWISPPPFMLNDTQVNTEYMVNAITALYAGSGNNKLPVLTWSQGGLVAQWGLTFFPSIRSKVDRLMAFAPDYKGTVLAGPLDALAVSAPSVWQQTTGSALTTALRNAGGLTQIVPTTNLYSATDEIVQPQVSNSPLDSSYLFNGKNVQAQAVCGPLFVIDHAGSLTSQFSYVVGRSALRSTTGQARSADYGITDCNPLPANDLTPEQKVAAAALLAPAAAAIVAGPKQNCEPDLMPYARPFAVGKRTCSGIVTP

SEQ ID NO: 2 - DNA, 957 bp, Pseudomonas putida
atgctgccgagtggcagtgacccggcgtttagtcagccgaagagcgtgctcgatgccggtctgacgtgtcaaggcgccagtccaagcagcgttagcaaaccgattctgctggttccgggcaccggtaccacgggcccgcagagcttcgacagcaactggattccgctgagtacccaactgggctacacgccgtgctggatcagtccaccaccgttcatgctgaacgacacccaagttaacacggagtacatggtgaatgcgatcaccgcgctgtacgccggcagtggtaacaataaactgccggtgctcacgtggagtcaaggcggtctggtggcccaatggggtctgaccttcttcccgagtatccgcagcaaagtggaccgtctgatggcgttcgccccggactacaaaggcaccgttctggccggtccactggatgcgctggccgttagtgccccgagcgtttggcagcagacgaccggtagtgcgctgaccaccgccctccgtaatgcgggtggtctgacccaaatcgtgccgacgaccaatctgtatagcgccacggacgagattgtgcagccacaagttagcaatagcccgctggacagcagctacctcttcaatggcaaaaacgtgcaagcccaagccgtttgtggtccgctgttcgttatcgatcacgccggtagtctgacgagccagttcagctatgtggttggtcgcagtgcgctgcgtagcaccaccggtcaagcccgtagcgccgattacggcattaccgactgcaacccgctgccagccaacgatctgaccccagaacagaaagttgcggccgcggcgctgctggcgccagccgcggccgccattgttgccggcccgaaacagaattgcgaaccggatctgatgccgtacgcgcgtccattcgccgtgggcaaacgcacgtgcagcggtattgttaccccgtaa